European Patent Application EP 4 338 748 A1, published March 20, 2024. Title: aggregation inhibitor for amiloid beta, medicament for disease by amiloid beta-aggregation and use therof. Applicant: O-Force Co., Ltd. The sequence listing filed with the application follows.

SEQUENCE LISTING (7 sequences)

SEQ ID NO: 1 - protein, 20 aa, Artificial Sequence
  aggregation inhibitor peptide
YKNMRETLVYLTHLDYDDTE

SEQ ID NO: 2 - protein, 5 aa, Artificial Sequence
  aggregation inhibitor peptide
YKNMR

SEQ ID NO: 3 - protein, 11 aa, Artificial Sequence
  aggregation inhibitor peptide
RETLVYLTHLD

SEQ ID NO: 4 - protein, 15 aa, Artificial Sequence
  aggregation inhibitor peptide
YKNMRETLVYLTHLD

SEQ ID NO: 5 - protein, 16 aa, Artificial Sequence
  aggregation inhibitor peptide
RETLVYLTHLDYDDTE

SEQ ID NO: 6 - protein, 42 aa, Homo sapiens [sequence omitted]

SEQ ID NO: 7 - protein, 11 aa, Homo sapiens
GSNKGAIIGLM